European Patent Specification EP 3 785 714 B1, published July 1, 2026. Title: PRODRUGS OF HIV REVERSE TRANSCRIPTASE INHIBITORS. Applicant: Merck Sharp & Dohme Corp. Burgey, Christopher S. Fritzen, Jeffrey F., Jr. Balsells, Jaume Patel, Mehul. The sequence listing filed with the application follows.

SEQUENCE LISTING (2 sequences)

SEQ ID NO: 1 - DNA, 21 bp, Artificial Sequence
  Chemically synthesized
ttgaaatgactgcggtacggc

SEQ ID NO: 2 - RNA, 501 nt, Artificial Sequence
  Chemically synthesized
gagguucaggugguuuccaccgcaacacaauccuuccuggcgaccugcgucaacggcguguguuggaccguuuaccauggugcuggcucaaagaccuuagccggcccaaaggggccaaucacccagauguacacuaauguggaccaggaccucgucggcuggcaggcgccccccggggcgcguuccuugacaccaugcaccuguggcagcucagaccuuuacuuggucacgagacaugcugacgucauuccggugcgccggcggggcgacaguagggggagccugcucucccccaggccugucuccuacuugaagggcucuucgggugguccacugcucugcccuucggggcacgcugugggcaucuuccgggcugccguaugcacccgggggguugcgaaggcgguggacuuugugcccguagaguccauggaaacuacuaugcggucuccggucuucacggacaacucaucccccccggccguaccgcagucauuucaa